European Patent Application EP 4 461 746 A2, published November 13, 2024. Title: ANTI-PD-1 AND ANTI-VEGFA BIFUNCTIONAL ANTIBODY, PHARMACEUTICAL COMPOSITION THEREOF AND USE THEREOF. Applicant: Akeso Biopharma, Inc. Application EP. The sequence listing filed with the application follows.

SEQUENCE LISTING (26 sequences)

SEQ ID NO: 1 - protein, 171 aa, synthetic construct
APMAEGGGQNHHEVVKFMDVYQRSYCHPIETLVDIFQEYPDEIEYIFKPSCVPLMRCGGCCNDEGLECVPTEESNITMQIMRIKPHQGQHIGEMSFLQHNKCECRPKKDRARQENPCGPCSERRKHLFVQDPQTCKCSCKNTDSRCKARQLELNERTCRCDKPRRHHHHHH

SEQ ID NO: 2 - DNA, 513 bp, synthetic construct
  source 1..513: mol_type = other DNA
gcacccatggccgagggcggcggccagaaccaccacgaggtggtgaagttcatggacgtgtaccagagaagctactgccaccccatcgagaccctggtggacatcttccaggagtaccccgacgagatcgagtacatcttcaagcccagctgcgtgcccctgatgagatgcggcggctgctgcaacgacgagggcctggagtgcgtgcccaccgaggagagcaacatcaccatgcagatcatgagaatcaagccccaccagggccagcacatcggcgagatgagcttcctgcagcacaacaagtgcgagtgcagacccaagaaggacagagccagacaggagaacccctgcggcccctgcagcgagagaagaaagcacctgttcgtgcaggacccccagacctgcaagtgcagctgcaagaacaccgacagcagatgcaaggccagacagctggagctgaacgagagaacctgcagatgcgacaagcccagaagacatcatcaccatcaccac

SEQ ID NO: 3 - protein, 998 aa, synthetic construct
MQSKVLLAVALWLCVETRAASVGLPSVSLDLPRLSIQKDILTIKANTTLQITCRGQRDLDWLWPNNQSGSEQRVEVTECSDGLFCKTLTIPKVIGNDTGAYKCFYRETDLASVIYVYVQDYRSPFIASVSDQHGVVYITENKNKTVVIPCLGSISNLNVSLCARYPEKRFVPDGNRISWDSKKGFTIPSYMISYAGMVFCEAKINDESYQSIMYIVVVVGYRIYDVVLSPSHGIELSVGEKLVLNCTARTELNVGIDFNWEYPSSKHQHKKLVNRDLKTQSGSEMKKFLSTLTIDGVTRSDQGLYTCAASSGLMTKKNSTFVRVHEKPFVAFGSGMESLVEATVGERVRIPAKYLGYPPPEIKWYKNGIPLESNHTIKAGHVLTIMEVSERDTGNYTVILTNPISKEKQSHVVSLVVYVPPQIGEKSLISPVDSYQYGTTQTLTCTVYAIPPPHHIHWYWQLEEECANEPSQAVSVTNPYPCEEWRSVEDFQGGNKIEVNKNQFALIEGKNKTVSTLVIQAANVSALYKCEAVNKVGRGERVISFHVTRGPEITLQPDMQPTEQESVSLWCTADRSTFENLTWYKLGPQPLPIHVGELPTPVCKNLDTLWKLNATMFSNSTNDILIMELKNASLQDQGDYVCLAQDRKTKKRHCVVRQLTVLERVAPTITGNLENQTTSIGESIEVSCTASGNPPPQIMWFKDNETLVEDSGIVLKDGNRNLTIRRVRKEDEGLYTCQACSVLGCAKVEAFFIIEGAQEKTNLESRENLYFQGTHTCPPCPAPELLGGPSVFLFPPKPKDTLMISRTPEVTCVVVDVSHEDPEVKFNWYVDGVEVHNAKTKPREEQYNSTYRVVSVLTVLHQDWLNGKEYKCKVSNKALPAPIEKTISKAKGQPREPQVYTLPPSRDELTKNQVSLTCLVKGFYPSDIAVEWESNGQPENNYKTTPPVLDSDGSFFLYSKLTVDKSRWQQGNVFSCSVMHEALHNHYTQKSLSLSPGK

SEQ ID NO: 4 - DNA, 2997 bp, synthetic construct
  source 1..2997: mol_type = other DNA
atgcagagcaaggtgctgctggccgtcgccctgtggctctgcgtggagacccgggccgcctctgtgggtttgcctagtgtttctcttgatctgcccaggctcagcatacaaaaagacatacttacaattaaggctaatacaactcttcaaattacttgcaggggacagagggacttggactggctttggcccaataatcagagtggcagtgagcaaagggtggaggtgactgagtgcagcgatggcctcttctgtaagacactcacaattccaaaagtgatcggaaatgacactggagcctacaagtgcttctaccgggaaactgacttggcctcggtcatttatgtctatgttcaagattacagatctccatttattgcttctgttagtgaccaacatggagtcgtgtacattactgagaacaaaaacaaaactgtggtgattccatgtctcgggtccatttcaaatctcaacgtgtcactttgtgcaagatacccagaaaagagatttgttcctgatggtaacagaatttcctgggacagcaagaagggctttactattcccagctacatgatcagctatgctggcatggtcttctgtgaagcaaaaattaatgatgaaagttaccagtctattatgtacatagttgtcgttgtagggtataggatttatgatgtggttctgagtccgtctcatggaattgaactatctgttggagaaaagcttgtcttaaattgtacagcaagaactgaactaaatgtggggattgacttcaactgggaatacccttcttcgaagcatcagcataagaaacttgtaaaccgagacctaaaaacccagtctgggagtgagatgaagaaatttttgagcaccttaactatagatggtgtaacccggagtgaccaaggattgtacacctgtgcagcatccagtgggctgatgaccaagaagaacagcacatttgtcagggtccatgaaaaaccttttgttgcttttggaagtggcatggaatctctggtggaagccacggtgggggagcgtgtcagaatccctgcgaagtaccttggttacccacccccagaaataaaatggtataaaaatggaataccccttgagtccaatcacacaattaaagcggggcatgtactgacgattatggaagtgagtgaaagagacacaggaaattacactgtcatccttaccaatcccatttcaaaggagaagcagagccatgtggtctctctggttgtgtatgtcccaccccagattggtgagaaatctctaatctctcctgtggattcctaccagtacggcaccactcaaacgctgacatgtacggtctatgccattcctcccccgcatcacatccactggtattggcagttggaggaagagtgcgccaacgagcccagccaagctgtctcagtgacaaacccatacccttgtgaagaatggagaagtgtggaggacttccagggaggaaataaaattgaagttaataaaaatcaatttgctctaattgaaggaaaaaacaaaactgtaagtacccttgttatccaagcggcaaatgtgtcagctttgtacaaatgtgaagcggtcaacaaagtcgggagaggagagagggtgatctccttccacgtgaccaggggtcctgaaattactttgcaacctgacatgcagcccactgagcaggagagcgtgtctttgtggtgcactgcagacagatctacgtttgagaacctcacatggtacaagcttggcccacagcctctgccaatccatgtgggagagttgcccacacctgtttgcaagaacttggatactctttggaaattgaatgccaccatgttctctaatagcacaaatgacattttgatcatggagcttaagaatgcatccttgcaggaccaaggagactatgtctgccttgctcaagacaggaagaccaagaaaagacattgcgtggtcaggcagctcacagtcctagagcgtgtggcacccacgatcacaggaaacctggagaatcagacgacaagtattggggaaagcatcgaagtctcatgcacggcatctgggaatccccctccacagatcatgtggtttaaagataatgagacccttgtagaagactcaggcattgtattgaaggatgggaaccggaacctcactatccgcagagtgaggaaggaggacgaaggcctctacacctgccaggcatgcagtgttcttggctgtgcaaaagtggaggcatttttcataatagaaggtgcccaggaaaagacgaacttggaatctagagaaaacctgtattttcagggcactcacacatgcccaccgtgcccagcacctgaactcctggggggaccgtcagtcttcctcttccccccaaaacccaaggacaccctcatgatctcccggacccctgaggtcacatgcgtggtggtggacgtgagccacgaagaccctgaggtcaagttcaactggtacgtggacggcgtggaggtgcataatgccaagacaaagccgcgggaggagcagtacaacagcacgtaccgtgtggtcagcgtcctcaccgtcctgcaccaggactggctgaatggcaaggagtacaagtgcaaggtctccaacaaagccctcccagcccccatcgagaaaaccatctccaaagccaaagggcagccccgagaaccacaggtgtacaccctgcccccatcccgggatgagctgaccaagaaccaggtcagcctgacctgcctggtcaaaggcttctatcccagcgacatcgccgtggagtgggagagcaatgggcagccggagaacaactacaagaccacgcctcccgtgttggactccgacggctccttcttcctctacagcaagctcaccgtggacaagagcaggtggcagcaggggaacgtcttctcatgctccgtgatgcatgaggctctgcacaaccactacacgcagaagagcctctccctgtctcccgggaaatga

SEQ ID NO: 5 - protein, 123 aa, synthetic construct [sequence omitted]

SEQ ID NO: 6 - DNA, 369 bp, synthetic construct
  source 1..369: mol_type = other DNA
gaggtgcagctggtcgagtccgggggggggctggtgcagccaggcgggtctctgaggctgagttgcgccgcttcagggtacaccttcacaaactatggaatgaattgggtgcgccaggcaccaggaaagggactggagtgggtcggctggatcaacacttacaccggggaacctacctatgcagccgactttaagcggcggttcaccttcagcctggatacaagcaaatccactgcctacctgcagatgaacagcctgcgagctgaggacaccgcagtctactattgtgctaaatatccccactactatgggagcagccattggtattttgacgtgtgggggcaggggactctggtgacagtgagcagc

SEQ ID NO: 7 - protein, 107 aa, synthetic construct [sequence omitted]

SEQ ID NO: 8 - DNA, 321 bp, synthetic construct
  source 1..321: mol_type = other DNA
gatattcagatgactcagagcccctcctccctgtccgcctctgtgggcgacagggtcaccatcacatgcagtgcttcacaggatatttccaactacctgaattggtatcagcagaagccaggaaaagcacccaaggtgctgatctacttcactagctccctgcactcaggagtgccaagccggttcagcggatccggatctggaaccgactttactctgaccatttctagtctgcagcctgaggatttcgctacatactattgccagcagtattctaccgtgccatggacatttggccaggggactaaagtcgagatcaag

SEQ ID NO: 9 - protein, 118 aa, synthetic construct
EVQLVESGGGLVQPGGSLRLSCAASGFAFSSYDMSWVRQAPGKGLDWVATISGGGRYTYYPDSVKGRFTISRDNSKNNLYLQMNSLRAEDTALYYCANRYGEAWFAYWGQGTLVTVSS

SEQ ID NO: 10 - DNA, 354 bp, synthetic construct
  source 1..354: mol_type = other DNA
gaagtgcagctggtcgagtctgggggagggctggtgcagcccggcgggtcactgcgactgagctgcgcagcttccggattcgcctttagctcctacgacatgtcctgggtgcgacaggcaccaggaaagggactggattgggtcgctactatctcaggaggcgggagatacacctactatcctgacagcgtcaagggccggttcacaatctctagagataacagtaagaacaatctgtatctgcagatgaacagcctgagggctgaggacaccgcactgtactattgtgccaaccgctacggggaagcatggtttgcctattgggggcagggaaccctggtgacagtctctagt

SEQ ID NO: 11 - protein, 107 aa, synthetic construct
DIQMTQSPSSMSASVGDRVTFTCRASQDINTYLSWFQQKPGKSPKTLIYRANRLVSGVPSRFSGSGSGQDYTLTISSLQPEDMATYYCLQYDEFPLTFGAGTKLELK

SEQ ID NO: 12 - DNA, 321 bp, synthetic construct
  source 1..321: mol_type = other DNA
gacattcagatgactcagagcccctcctccatgtccgcctctgtgggcgacagggtcaccttcacatgccgcgctagtcaggatatcaacacctacctgagctggtttcagcagaagccagggaaaagccccaagacactgatctaccgggctaatagactggtgtctggagtcccaagtcggttcagtggctcagggagcggacaggactacactctgaccatcagctccctgcagcctgaggacatggcaacctactattgcctgcagtatgatgagttcccactgacctttggcgccgggacaaaactggagctgaag

SEQ ID NO: 13 - protein, 20 aa, synthetic construct
GGGGSGGGGSGGGGSGGGGS

SEQ ID NO: 14 - protein, 5 aa, synthetic construct
GGGGS

SEQ ID NO: 15 - protein, 8 aa, synthetic construct
GYTFTNYG

SEQ ID NO: 16 - protein, 8 aa, synthetic construct
INTYTGEP

SEQ ID NO: 17 - protein, 16 aa, synthetic construct
AKYPHYYGSSHWYFDV

SEQ ID NO: 18 - protein, 6 aa, synthetic construct
QDISNY

SEQ ID NO: 19 - skipped

SEQ ID NO: 20 - protein, 9 aa, synthetic construct
QQYSTVPWT

SEQ ID NO: 21 - protein, 8 aa, synthetic construct
GFAFSSYD

SEQ ID NO: 22 - protein, 8 aa, synthetic construct
ISGGGRYT

SEQ ID NO: 23 - protein, 11 aa, synthetic construct
ANRYGEAWFAY

SEQ ID NO: 24 - protein, 6 aa, synthetic construct
QDINTY

SEQ ID NO: 25 - skipped

SEQ ID NO: 26 - protein, 9 aa, synthetic construct
LQYDEFPLT